European Patent Application EP 4 130 289 A1, published February 8, 2023. Title: Method and program of calculating methylation level of a base. Applicant: FUJIFILM Corporation. The sequence listing filed with the application follows.

SEQUENCE LISTING (6 sequences)

SEQ ID NO: 1 - DNA, 99 bp, Enterobacteria phage lambda
  Partial DNA of Enterobacteria phage lambda DNA
ttgatggtattgcacagaatatggcggcgatgctgaccggcagtgagcagaactggcgcagcttcacccgttccgtgctgtccatgatgacagaaattc

SEQ ID NO: 2 - DNA, 24 bp, Artificial Sequence
  Forward primer
ttgatggtattgtatagaatatgg

SEQ ID NO: 3 - DNA, 24 bp, Artificial Sequence
  Reverse primer
aaatttctatcatcataaacaaca

SEQ ID NO: 4 - DNA, 10 bp, Artificial Sequence
  Example of molecular barcode
atgatcgatc

SEQ ID NO: 5 - DNA, 10 bp, Artificial Sequence
  Example of molecular barcode
ctgatccaat

SEQ ID NO: 6 - DNA, 99 bp, Artificial Sequence
  Example of read
ttgatggtattgtatagaatatggcggcgatgttgatcggtagtgagtagaattggcgtagttttattcgtttcgtgttgtttatgatgatagaaattt